European Patent Application EP 4 296 279 A1, published December 27, 2023. Title: Anti-transthyretin (TTR) binding proteins and uses thereof. Applicant: Fraunhofer-Gesellschaft zur Förderung der angewandten Forschung e.V. The sequence listing filed with the application follows.

SEQUENCE LISTING (38 sequences)

SEQ ID NO: 1 - protein, 127 aa, Artificial Sequence
  human transthyretin
GPTGTGESKCPLMVKVLDAVRGSPAINVAVHVFRKAADDTWEPFASGKTSESGELHGLTTEEEFVEGIYKVEIDTKSYWKALGISPFHEHAEVVFTANDSGPRRYTIAALLSPYSYSTTAVVTNPKE

SEQ ID NO: 2 - protein, 9 aa, Artificial Sequence
  residues 35-43 of transthyretin
KAADDTWEP

SEQ ID NO: 3 - protein, 9 aa, Artificial Sequence
  isoD38 TTR (35-43)
  MOD_RES 4: L-isoaspartate
KAAXDTWEP

SEQ ID NO: 4 - protein, 10 aa, Artificial Sequence
  isoD38 TTR (35-43)Cys
  MOD_RES 4: L-isoaspartate
KAAXDTWEPC

SEQ ID NO: 5 - protein, 9 aa, Artificial Sequence
  MOD_RES 1: PEG-biotin
  isoD38 TTR (35-43)PEG-Biotin
  MOD_RES 4: L-isoaspartate
  MOD_RES 9: amidated
KAAXDTWEP

SEQ ID NO: 6 - protein, 9 aa, Artificial Sequence
  MOD_RES 1: PEG-Biotin
  TTR (35-43)PEG-Biotin
  MOD_RES 9: amidated
KAADDTWEP

SEQ ID NO: 7 - protein, 127 aa, Artificial Sequence
  human transthyretin with V30M substitution
GPTGTGESKCPLMVKVLDAVRGSPAINVAMHVFRKAADDTWEPFASGKTSESGELHGLTTEEEFVEGIYKVEIDTKSYWKALGISPFHEHAEVVFTANDSGPRRYTIAALLSPYSYSTTAVVTNPKE

SEQ ID NO: 8 - protein, 127 aa, Artificial Sequence
  human transthyretin with V122I substitution
GPTGTGESKCPLMVKVLDAVRGSPAINVAVHVFRKAADDTWEPFASGKTSESGELHGLTTEEEFVEGIYKVEIDTKSYWKALGISPFHEHAEVVFTANDSGPRRYTIAALLSPYSYSTTAVITNPKE

SEQ ID NO: 9 - protein, 42 aa, Artificial Sequence [sequence omitted]

SEQ ID NO: 10 - protein, 42 aa, Artificial Sequence
  amyloid beta (1-42) with L-isoaspartate at position 7
  MOD_RES 7: L-isoaspartate
DAEFRHXSGYEVHHQKLVFFAEDVGSNKGAIIGLMVGGVVIA

SEQ ID NO: 11 - protein, 17 aa, Artificial Sequence
  2F2 LCDR1
KSSQSVLYSSNQKNYLA

SEQ ID NO: 12 - protein, 7 aa, Artificial Sequence
  2F2 LCDR2
WASTRES

SEQ ID NO: 13 - protein, 8 aa, Artificial Sequence
  2F2 LCDR3
HQYLSSRT

SEQ ID NO: 14 - protein, 10 aa, Artificial Sequence
  2F2 HCDR1
GFTFSSFAMH

SEQ ID NO: 15 - protein, 17 aa, Artificial Sequence
  2F2 HCDR2
FISSGSNTIYYADTVKG

SEQ ID NO: 16 - protein, 8 aa, Artificial Sequence
  2F2 HCDR3
NSYYGMDY

SEQ ID NO: 17 - protein, 112 aa, Artificial Sequence
  2F2 VL
NIMMTQSPSSLAVSAGEKVTMSCKSSQSVLYSSNQKNYLAWYQQKPGQSPKLLIYWASTRESGVPDRFTGSGSGTDFTLTISSVQAEDLAVYYCHQYLSSRTFGAGTKLELK

SEQ ID NO: 18 - protein, 117 aa, Artificial Sequence
  2F2 VH
DVQLVESGGGLVQPGGSRKLSCAASGFTFSSFAMHWVRQAPDKGLEWVAFISSGSNTIYYADTVKGRFTVSRDNPKNTLFLQMTSLRSEDTAMYYCASNSYYGMDYWGQGTSVTVSS

SEQ ID NO: 19 - DNA, 336 bp, Artificial Sequence
  2F2 VL DNA
aacattatgatgacgcagtcgccatcatctctggctgtgtctgcaggagaaaaggtcactatgagctgtaagtccagtcagagtgttttatacagttcaaatcagaagaattacttggcctggtaccagcagaaaccagggcagtctcctaaactgctgatctactgggcatccactagggaatctggtgtccctgatcgcttcacaggcagtggatctgggacagattttactctcaccatcagcagtgtacaagctgaagacctggcagtttattactgtcatcaatacctctcctcgcgcacgttcggtgctgggaccaagctggagctgaag

SEQ ID NO: 20 - DNA, 351 bp, Artificial Sequence
  2F2 VH DNA
gatgtgcagctggtggagtctgggggaggcttagtgcagcctggagggtcccggaaactctcctgtgcagcctctggattcactttcagtagctttgcaatgcactgggttcgtcaggctccagacaaggggctggagtgggtcgcattcattagtagtggcagtaataccatctactatgcagacacagtgaagggccgattcaccgtctccagagacaatcccaagaacaccctgttcctgcaaatgaccagtctaaggtctgaggacacggccatgtattactgtgcaagtaattcgtactatggtatggactactggggtcaaggaacctcagtcaccgtctcctca

SEQ ID NO: 21 - protein, 11 aa, Artificial Sequence
  4D4 LCDR1
RTSGNIRNSLA

SEQ ID NO: 22 - protein, 7 aa, Artificial Sequence
  4D4 LCDR2
NGKTLAD

SEQ ID NO: 23 - protein, 9 aa, Artificial Sequence
  4D4 LCDR3
QHFWNIPFT

SEQ ID NO: 24 - protein, 10 aa, Artificial Sequence
  4D4 HCDR1
GNTFSSRWIE

SEQ ID NO: 25 - protein, 17 aa, Artificial Sequence
  4D4 HCDR2
EIFPGNGNTNYNEKFKG

SEQ ID NO: 26 - skipped

SEQ ID NO: 27 - protein, 107 aa, Artificial Sequence
  4D4 VL
DIQMTQSPASLSASVGETVTITCRTSGNIRNSLAWYRQKQGKSPQLLVFNGKTLADGVPSRFSGSGSGTQYSLKINSLQPEDLGTYYCQHFWNIPFTFGSGTKLEIK

SEQ ID NO: 28 - protein, 112 aa, Artificial Sequence
  4D4 VH
QVQLQQSGAELMKPGASVKISCKAPGNTFSSRWIEWVKERPGHGLEWIGEIFPGNGNTNYNEKFKGKATFTADTSSNTAYIQFSSLASEDSGVYYCVSEDYWGQGTLVTVSS

SEQ ID NO: 29 - DNA, 321 bp, Artificial Sequence
  4D4 VL DNA
gacatccagatgactcagtctccagcctccctatctgcatctgtgggagaaactgtcaccatcacatgtcgaacaagtgggaatattcgcaattcattagcatggtatcgacagaaacagggaaaatcccctcagctcctggtctttaatggcaaaactttagcagatggtgtgccatcaaggttcagtggcagtggatcaggaacacaatattctctcaagatcaacagcctgcagcctgaagatttagggacttattactgtcaacatttttggaatattccattcacgttcggctcggggacaaagttggaaataaaa

SEQ ID NO: 30 - DNA, 336 bp, Artificial Sequence
  4D4 VH DNA
caggttcagctgcagcagtctggagctgagctgatgaagcctggggcctcagtgaagatatcctgcaaggctcctggcaacacattcagtagcaggtggatagagtgggtaaaggagaggcctggacatggccttgagtggattggagagatttttcctggaaatggtaatactaactacaatgagaagttcaagggcaaggccacattcactgcagatacatcctccaacacagcctatatacaattcagcagcctggcatctgaggactctggcgtctattactgtgtatctgaagactattggggccaaggtaccctggtcaccgtctcctca

SEQ ID NO: 31 - protein, 219 aa, Artificial Sequence
  2F2 LC
NIMMTQSPSSLAVSAGEKVTMSCKSSQSVLYSSNQKNYLAWYQQKPGQSPKLLIYWASTRESGVPDRFTGSGSGTDFTLTISSVQAEDLAVYYCHQYLSSRTFGAGTKLELKRADAAPTVSIFPPSSEQLTSGGASVVCFLNNFYPKDINVKWKIDGSERQNGVLNSWTDQDSKDSTYSMSSTLTLTKDEYERHNSYTCEATHKTSTSPIVKSFNRNEC

SEQ ID NO: 32 - protein, 447 aa, Artificial Sequence
  2F2 HC
DVQLVESGGGLVQPGGSRKLSCAASGFTFSSFAMHWVRQAPDKGLEWVAFISSGSNTIYYADTVKGRFTVSRDNPKNTLFLQMTSLRSEDTAMYYCASNSYYGMDYWGQGTSVTVSSATTTAPSVYPLVPGCSDTSGSSVTLGCLVKGYFPEPVTVKWNYGALSSGVRTVSSVLQSGFYSLSSLVTVPSSTWPSQTVICNVAHPASKTELIKRIEPRIPKPSTPPGSSCPPGNILGGPSVFIFPPKPKDALMISLTPKVTCVVVDVSEDDPDVHVSWFVDNKEVHTAWTQPREAQYNSTFRVVSALPIQHQDWMRGKEFKCKVNNKALPAPIERTISKPKGRAQTPQVYTIPPPREQMSKKKVSLTCLVTNFFSEAISVEWERNGELEQDYKNTPPILDSDGTYFLYSKLTVDTDSWLQGEIFTCSVVHEALHNHHTQKNLSRSPGK

SEQ ID NO: 33 - protein, 214 aa, Artificial Sequence
  4D4 LC
DIQMTQSPASLSASVGETVTITCRTSGNIRNSLAWYRQKQGKSPQLLVFNGKTLADGVPSRFSGSGSGTQYSLKINSLQPEDLGTYYCQHFWNIPFTFGSGTKLEIKRADAAPTVSIFPPSSEQLTSGGASVVCFLNNFYPKDINVKWKIDGSERQNGVLNSWTDQDSKDSTYSMSSTLTLTKDEYERHNSYTCEATHKTSTSPIVKSFNRNEC

SEQ ID NO: 34 - protein, 442 aa, Artificial Sequence
  4D4 HC
QVQLQQSGAELMKPGASVKISCKAPGNTFSSRWIEWVKERPGHGLEWIGEIFPGNGNTNYNEKFKGKATFTADTSSNTAYIQFSSLASEDSGVYYCVSEDYWGQGTLVTVSSAKTTAPSVYPLAPVCGDTTGSSVTLGCLVKGYFPEPVTLTWNSGSLSSGVHTFPAVLQSDLYTLSSSVTVTSSTWPSQSITCNVAHPASSTKVDKKIEPRGPTIKPCPPCKCPAPNLLGGPSVFIFPPKIKDVLMISLSPIVTCVVVDVSEDDPDVQISWFVNNVEVHTAQTQTHREDYNSTLRVVSALPIQHQDWMSGKEFKCKVNNKDLPAPIERTISKPKGSVRAPQVYVLPPPEEEMTKKQVTLTCMVTDFMPEDIYVEWTNNGKTELNYKNTEPVLDSDGSYFMYSKLRVEKKNWVERNSYSCSVVHEGLHNHHTTKSFSRTPGK

SEQ ID NO: 35 - DNA, 660 bp, Artificial Sequence
  2F2 LC
aacattatgatgacgcagtcgccatcatctctggctgtgtctgcaggagaaaaggtcactatgagctgtaagtccagtcagagtgttttatacagttcaaatcagaagaattacttggcctggtaccagcagaaaccagggcagtctcctaaactgctgatctactgggcatccactagggaatctggtgtccctgatcgcttcacaggcagtggatctgggacagattttactctcaccatcagcagtgtacaagctgaagacctggcagtttattactgtcatcaatacctctcctcgcgcacgttcggtgctgggaccaagctggagctgaagcgggctgatgctgcaccaactgtatccatcttcccaccatccagtgagcagttaacatctggaggtgcctcagtcgtgtgcttcttgaacaacttctaccccaaagacatcaatgtcaagtggaagattgatggcagtgaacgacaaaatggcgtcctgaacagttggactgatcaggacagcaaagacagcacctacagcatgagcagcaccctcacgttgaccaaggacgagtatgaacgacataacagctatacctgtgaggccactcacaagacatcaacttcacccattgtcaagagcttcaacaggaatgagtgttag

SEQ ID NO: 36 - DNA, 1341 bp, Artificial Sequence
  2F2 HC
gatgtgcagctggtggagtctgggggaggcttagtgcagcctggagggtcccggaaactctcctgtgcagcctctggattcactttcagtagctttgcaatgcactgggttcgtcaggctccagacaaggggctggagtgggtcgcattcattagtagtggcagtaataccatctactatgcagacacagtgaagggccgattcaccgtctccagagacaatcccaagaacaccctgttcctgcaaatgaccagtctaaggtctgaggacacggccatgtattactgtgcaagtaattcgtactatggtatggactactggggtcaaggaacctcagtcaccgtctcctcagctacaacaacagccccatctgtctatcccttggtccctggctgcagtgacacatctggatcctcggtgacactgggatgccttgtcaaaggctacttccctgagccggtaactgtaaaatggaactatggagccctgtccagcggtgtgcgcacagtctcatctgtcctgcagtctgggttctattccctcagcagcttggtgactgtaccctccagcacctggcccagccagactgtcatctgcaacgtagcccacccagccagcaagactgagttgatcaagagaatcgagcctagaatacccaagcccagtacccccccaggttcttcatgcccacctggtaacatcttgggtggaccatccgtcttcatcttccccccaaagcccaaggatgcactcatgatctccctaacccccaaggttacgtgtgtggtggtggatgtgagcgaggatgacccagatgtccatgtcagctggtttgtggacaacaaagaagtacacacagcctggacacagccccgtgaagctcagtacaacagtaccttccgagtggtcagtgccctccccatccagcaccaggactggatgaggggcaaggagttcaaatgcaaggtcaacaacaaagccctcccagcccccatcgagagaaccatctcaaaacccaaaggaagagcccagacacctcaagtatacaccatacccccacctcgtgaacaaatgtccaagaagaaggttagtctgacctgcctggtcaccaacttcttctctgaagccatcagtgtggagtgggaaaggaacggagaactggagcaggattacaagaacactccacccatcctggactcagatgggacctacttcctctacagcaagctcactgtggatacagacagttggttgcaaggagaaatttttacctgctccgtggtgcatgaggctctccataaccaccacacacagaagaacctgtctcgctcccctggtaaa

SEQ ID NO: 37 - DNA, 645 bp, Artificial Sequence
  4D4 LC
gacatccagatgactcagtctccagcctccctatctgcatctgtgggagaaactgtcaccatcacatgtcgaacaagtgggaatattcgcaattcattagcatggtatcgacagaaacagggaaaatcccctcagctcctggtctttaatggcaaaactttagcagatggtgtgccatcaaggttcagtggcagtggatcaggaacacaatattctctcaagatcaacagcctgcagcctgaagatttagggacttattactgtcaacatttttggaatattccattcacgttcggctcggggacaaagttggaaataaaacgggctgatgctgcaccaactgtatccatcttcccaccatccagtgagcagttaacatctggaggtgcctcagtcgtgtgcttcttgaacaacttctaccccaaagacatcaatgtcaagtggaagattgatggcagtgaacgacaaaatggcgtcctgaacagttggactgatcaggacagcaaagacagcacctacagcatgagcagcaccctcacgttgaccaaggacgagtatgaacgacataacagctatacctgtgaggccactcacaagacatcaacttcacccattgtcaagagcttcaacaggaatgagtgttag

SEQ ID NO: 38 - DNA, 1329 bp, Artificial Sequence
  4D4 HC
caggttcagctgcagcagtctggagctgagctgatgaagcctggggcctcagtgaagatatcctgcaaggctcctggcaacacattcagtagcaggtggatagagtgggtaaaggagaggcctggacatggccttgagtggattggagagatttttcctggaaatggtaatactaactacaatgagaagttcaagggcaaggccacattcactgcagatacatcctccaacacagcctatatacaattcagcagcctggcatctgaggactctggcgtctattactgtgtatctgaagactattggggccaaggtaccctggtcaccgtctcctcagccaagaccaccgcccccagcgtgtaccctctggctcctgtgtgtggcgataccaccggcagctctgtgaccctgggctgcctcgtgaagggatacttccccgagccagtgaccctgacctggaacagcggctctctgagcagcggagtgcacacctttccagccgtgctgcagagcgacctgtacaccctgagcagcagcgtgaccgtgacctccagcacatggcccagccagagcatcacctgtaacgtggcccaccctgccagcagcaccaaggtggacaagaagatcgagcccagaggccccaccatcaagccttgccccccttgcaaatgccctgcccccaatctgctgggcggaccctccgtgtttatcttcccacccaagatcaaggacgtgctgatgatcagcctgagccccatcgtgacctgcgtggtggtggacgtgtccgaggacgaccccgatgtgcagatcagttggttcgtgaacaacgtggaagtgcacacagcccagacccagacacacagagaggactacaacagcaccctgagggtggtgtccgccctgcctatccagcaccaggattggatgagcggcaaagaattcaagtgcaaagtgaacaacaaggacctgccagcccccatcgagcggaccatctctaagcctaagggcagcgtgcgggctccccaggtgtacgtgctgcctcctccagaggaagagatgaccaagaaacaagtgacactgacatgcatggtcaccgacttcatgcccgaggacatctacgtggaatggaccaacaacggcaagaccgagctgaactacaagaataccgagcccgtgctggacagcgacggcagctacttcatgtacagcaagctgcgggtggaaaagaaaaactgggtggaacggaacagctacagctgcagcgtggtgcacgagggcctgcacaatcaccacaccaccaagagcttcagccggacccccggcaaatga